European Patent Specification EP 3 303 627 B1, published December 11, 2024. Title: COMPOSITIONS, SYSTEMS, AND METHODS FOR SEQUENCING POLYNUCLEOTIDES USING TETHERS ANCHORED TO POLYMERASES ADJACENT TO NANOPORES. Applicant: ILLUMINA, INC. Application EP 16730141.5. The sequence listing filed with the application follows.

SEQUENCE LISTING (1 sequence)

SEQ ID NO: 1 - DNA, 26 bp, Artificial Sequence
  source: /note="Description of Artificial Sequence: Synthetic oligonucleotide"
  misc_feature (12)..(12): n = one or more abasic nucleotides
  misc_feature (26)..(26): 3' maleimide group
tttttttttttntttttttatatggg